European Patent Application EP 4 541 823 A1, published April 23, 2025. Title: Phase Change Adjusting Element and Use Thereof. Applicant: Tsinghua University. Application IB PCT/CN2023/000077, filed June 16, 2023. The sequence listing filed with the application follows.

SEQUENCE LISTING (28 sequences)

SEQ ID NO: 1 - protein, 607 aa, synthetic construct
  REGION 1..607: note = PRM SH3 N C MBP His6
  source 1..607: note = Tandem repeats of the PRM domain and SH3 domain, with an MBP tag fused to the N-terminal and a His6 tag fused to the C-terminal, respectively.
MKIEEGKLVIWINGDKGYNGLAEVGKKFEKDTGIKVTVEHPDKLEEKFPQVAATGDGPDIIFWAHDRFGGYAQSGLLAEITPDKAFQDKLYPFTWDAVRYNGKLIAYPIAVEALSLIYNKDLLPNPPKTWEEIPALDKELKAKGKSALMFNLQEPYFTWPLIAADGGYAFKYENGKYDIKDVGVDNAGAKAGLTFLVDLIKNKHMNADTDYSIAEAAFNKGETAMTINGPWAWSNIDTSKVNYGVTVLPTFKGQPSKPFVGVLSAGINAASPNKELAKEFLENYLLTDEGLEAVNKDKPLGAVALKSYEEELVKDPRIAATMENAQKGEIMPNIPQMSAFWYAVRTAVINAASGRQTVDEALKDAQTNSSSENLYFQGGSGSASMKGGSWGGSKKTPPPVPPRTTSKGGSGGSGGSGGSKKTPPPVPPRTTSKGGSGGSGGSGGSDLNMPAYVKFNYMAEREDELSLIKGTKVIVMEKSSDGWWRGSYNGQVGWFPSNYVTEEGDSPLASGAGGSEGGGSEGGTSGATDLNMPAYVKFNYMAEREDELSLIKGTKVIVMEKSSDGWWRGSYNGQVGWFPSNYVTEEGDSPLGSMGEFPAGNHHHHHH

SEQ ID NO: 2 - protein, 520 aa, synthetic construct
  REGION 1..520: note = CXCR4 N C MBP His6
  source 1..520: note = Anti-CXCR4 nanobody, with MBP tag and His6 tag fused to the N-terminal and C-terminal respectively
MKIEEGKLVIWINGDKGYNGLAEVGKKFEKDTGIKVTVEHPDKLEEKFPQVAATGDGPDIIFWAHDRFGGYAQSGLLAEITPDKAFQDKLYPFTWDAVRYNGKLIAYPIAVEALSLIYNKDLLPNPPKTWEEIPALDKELKAKGKSALMFNLQEPYFTWPLIAADGGYAFKYENGKYDIKDVGVDNAGAKAGLTFLVDLIKNKHMNADTDYSIAEAAFNKGETAMTINGPWAWSNIDTSKVNYGVTVLPTFKGQPSKPFVGVLSAGINAASPNKELAKEFLENYLLTDEGLEAVNKDKPLGAVALKSYEEELVKDPRIAATMENAQKGEIMPNIPQMSAFWYAVRTAVINAASGRQTVDEALKDAQTNSSSENLYFQGGSEVQLMESGGGLVQAGGSLRLSCAASGRTFNNYAMGWFRRAPKGEREFVAAITRSGVRSGVSAIYGDSVKDRFTISRDNAKNTLYLQMNSLKPEDTAVYTCAASAIGSGALRRFEYDYSGQGTQVTVSSEFPAGNHHHHHH

SEQ ID NO: 3 - protein, 516 aa, synthetic construct
  REGION 1..516: note = DR5 N C MBP His6
  source 1..516: note = Anti-DR5 nanobody, with MBP tag and His6 tag fused to the N-terminal and C-terminal respectively
MKIEEGKLVIWINGDKGYNGLAEVGKKFEKDTGIKVTVEHPDKLEEKFPQVAATGDGPDIIFWAHDRFGGYAQSGLLAEITPDKAFQDKLYPFTWDAVRYNGKLIAYPIAVEALSLIYNKDLLPNPPKTWEEIPALDKELKAKGKSALMFNLQEPYFTWPLIAADGGYAFKYENGKYDIKDVGVDNAGAKAGLTFLVDLIKNKHMNADTDYSIAEAAFNKGETAMTINGPWAWSNIDTSKVNYGVTVLPTFKGQPSKPFVGVLSAGINAASPNKELAKEFLENYLLTDEGLEAVNKDKPLGAVALKSYEEELVKDPRIAATMENAQKGEIMPNIPQMSAFWYAVRTAVINAASGRQTVDEALKDAQTNSSSENLYFQGGSMGEVQLLESGGGLVQPGGSLRLSCAASGTFDKINNMGWYRQAPGKQRDLVAQITPGGITDYADSVKGRFTISRDNSKNTLYLQMNSLRPEDTAVYYCNAEILKRAYIDVYVNYWGQGTLVTVSSEFPAGNHHHHHH

SEQ ID NO: 4 - protein, 519 aa, synthetic construct
  REGION 1..519: note = EGFR N C MBP His6
  source 1..519: note = Anti-EGFR nanobody, with MBP tag and His6 tag fused to the N-terminal and C-terminal respectively
MKIEEGKLVIWINGDKGYNGLAEVGKKFEKDTGIKVTVEHPDKLEEKFPQVAATGDGPDIIFWAHDRFGGYAQSGLLAEITPDKAFQDKLYPFTWDAVRYNGKLIAYPIAVEALSLIYNKDLLPNPPKTWEEIPALDKELKAKGKSALMFNLQEPYFTWPLIAADGGYAFKYENGKYDIKDVGVDNAGAKAGLTFLVDLIKNKHMNADTDYSIAEAAFNKGETAMTINGPWAWSNIDTSKVNYGVTVLPTFKGQPSKPFVGVLSAGINAASPNKELAKEFLENYLLTDEGLEAVNKDKPLGAVALKSYEEELVKDPRIAATMENAQKGEIMPNIPQMSAFWYAVRTAVINAASGRQTVDEALKDAQTNSSSENLYFQGGSEVQLVESGGGLVQAGGSLRLSCAASGRTFSSYAMGWFRQAPGKEREFVVAINWSSGSTYYADSVKGRFTISRDNAKNTMYLQMNSLKPEDTAVYYCAAGYQINSGNYNFKDYEYDYWGQGTQVTVSSEFPAGNHHHHHH

SEQ ID NO: 5 - protein, 508 aa, synthetic construct
  REGION 1..508: note = C-Met N C MBP His6
  source 1..508: note = Anti-C-Met nanobody, with MBP tag and His6 tag fused to the N-terminal and C-terminal respectively
MKIEEGKLVIWINGDKGYNGLAEVGKKFEKDTGIKVTVEHPDKLEEKFPQVAATGDGPDIIFWAHDRFGGYAQSGLLAEITPDKAFQDKLYPFTWDAVRYNGKLIAYPIAVEALSLIYNKDLLPNPPKTWEEIPALDKELKAKGKSALMFNLQEPYFTWPLIAADGGYAFKYENGKYDIKDVGVDNAGAKAGLTFLVDLIKNKHMNADTDYSIAEAAFNKGETAMTINGPWAWSNIDTSKVNYGVTVLPTFKGQPSKPFVGVLSAGINAASPNKELAKEFLENYLLTDEGLEAVNKDKPLGAVALKSYEEELVKDPRIAATMENAQKGEIMPNIPQMSAFWYAVRTAVINAASGRQTVDEALKDAQTNSSSEVQLVESGGGLVQPGGSLRLSCAASGFILDYYAIGWFRQAPGKEREGVLCIDASDDITYYADSVKGRFTISRDNAKNTVYLQMNSLKPEDTGVYYCATPIGLSSSCLLEYDYDYWGQGTLVTVSSEFPAGNHHHHHH

SEQ ID NO: 6 - protein, 663 aa, synthetic construct
MKIEEGKLVIWINGDKGYNGLAEVGKKFEKDTGIKVTVEHPDKLEEKFPQVAATGDGPDIIFWAHDRFGGYAQSGLLAEITPDKAFQDKLYPFTWDAVRYNGKLIAYPIAVEALSLIYNKDLLPNPPKTWEEIPALDKELKAKGKSALMFNLQEPYFTWPLIAADGGYAFKYENGKYDIKDVGVDNAGAKAGLTFLVDLIKNKHMNADTDYSIAEAAFNKGETAMTINGPWAWSNIDTSKVNYGVTVLPTFKGQPSKPFVGVLSAGINAASPNKELAKEFLENYLLTDEGLEAVNKDKPLGAVALKSYEEELVKDPRIAATMENAQKGEIMPNIPQMSAFWYAVRTAVINAASGRQTVDEALKDAQTNSSSENLYFQGGSEVQLMESGGGLVQAGGSLRLSCAASGRTFNNYAMGWFRRAPKGEREFVAAITRSGVRSGVSAIYGDSVKDRFTISRDNAKNTLYLQMNSLKPEDTAVYTCAASAIGSGALRRFEYDYSGQGTQVTVSSGGSGGSGGSGGSASSRSMGMGEVQLLESGGGLVQPGGSLRLSCAASGTFDKINNMGWYRQAPGKQRDLVAQITPGGITDYADSVKGRFTISRDNSKNTLYLQMNSLRPEDTAVYYCNAEILKRAYIDVYVNYWGQGTLVTVSSEFPAGNHHHHHH

SEQ ID NO: 7 - protein, 869 aa, synthetic construct
MKIEEGKLVIWINGDKGYNGLAEVGKKFEKDTGIKVTVEHPDKLEEKFPQVAATGDGPDIIFWAHDRFGGYAQSGLLAEITPDKAFQDKLYPFTWDAVRYNGKLIAYPIAVEALSLIYNKDLLPNPPKTWEEIPALDKELKAKGKSALMFNLQEPYFTWPLIAADGGYAFKYENGKYDIKDVGVDNAGAKAGLTFLVDLIKNKHMNADTDYSIAEAAFNKGETAMTINGPWAWSNIDTSKVNYGVTVLPTFKGQPSKPFVGVLSAGINAASPNKELAKEFLENYLLTDEGLEAVNKDKPLGAVALKSYEEELVKDPRIAATMENAQKGEIMPNIPQMSAFWYAVRTAVINAASGRQTVDEALKDAQTNSSSENLYFQGGSEVQLMESGGGLVQAGGSLRLSCAASGRTFNNYAMGWFRRAPKGEREFVAAITRSGVRSGVSAIYGDSVKDRFTISRDNAKNTLYLQMNSLKPEDTAVYTCAASAIGSGALRRFEYDYSGQGTQVTVSSGGSGGSGGSGGSASMKGGSWGGSKKTPPPVPPRTTSKGGSGGSGGSGGSKKTPPPVPPRTTSKGGSGGSGGSGGSDLNMPAYVKFNYMAEREDELSLIKGTKVIVMEKSSDGWWRGSYNGQVGWFPSNYVTEEGDSPLASGAGGSEGGGSEGGTSGATDLNMPAYVKFNYMAEREDELSLIKGTKVIVMEKSSDGWWRGSYNGQVGWFPSNYVTEEGDSPLGSMGMGEVQLLESGGGLVQPGGSLRLSCAASGTFDKINNMGWYRQAPGKQRDLVAQITPGGITDYADSVKGRFTISRDNSKNTLYLQMNSLRPEDTAVYYCNAEILKRAYIDVYVNYWGQGTLVTVSSEFPAGNHHHHHH

SEQ ID NO: 8 - protein, 868 aa, synthetic construct
MKIEEGKLVIWINGDKGYNGLAEVGKKFEKDTGIKVTVEHPDKLEEKFPQVAATGDGPDIIFWAHDRFGGYAQSGLLAEITPDKAFQDKLYPFTWDAVRYNGKLIAYPIAVEALSLIYNKDLLPNPPKTWEEIPALDKELKAKGKSALMFNLQEPYFTWPLIAADGGYAFKYENGKYDIKDVGVDNAGAKAGLTFLVDLIKNKHMNADTDYSIAEAAFNKGETAMTINGPWAWSNIDTSKVNYGVTVLPTFKGQPSKPFVGVLSAGINAASPNKELAKEFLENYLLTDEGLEAVNKDKPLGAVALKSYEEELVKDPRIAATMENAQKGEIMPNIPQMSAFWYAVRTAVINAASGRQTVDEALKDAQTNSSSENLYFQGGSEVQLVESGGGLVQAGGSLRLSCAASGRTFSSYAMGWFRQAPGKEREFVVAINWSSGSTYYADSVKGRFTISRDNAKNTMYLQMNSLKPEDTAVYYCAAGYQINSGNYNFKDYEYDYWGQGTQVTVSSGGSGGSGGSGGSASMKGGSWGGSKKTPPPVPPRTTSKGGSGGSGGSGGSKKTPPPVPPRTTSKGGSGGSGGSGGSDLNMPAYVKFNYMAEREDELSLIKGTKVIVMEKSSDGWWRGSYNGQVGWFPSNYVTEEGDSPLASGAGGSEGGGSEGGTSGATDLNMPAYVKFNYMAEREDELSLIKGTKVIVMEKSSDGWWRGSYNGQVGWFPSNYVTEEGDSPLGSMGMGEVQLLESGGGLVQPGGSLRLSCAASGTFDKINNMGWYRQAPGKQRDLVAQITPGGITDYADSVKGRFTISRDNSKNTLYLQMNSLRPEDTAVYYCNAEILKRAYIDVYVNYWGQGTLVTVSSEFPAGNHHHHHH

SEQ ID NO: 9 - protein, 866 aa, synthetic construct
MKIEEGKLVIWINGDKGYNGLAEVGKKFEKDTGIKVTVEHPDKLEEKFPQVAATGDGPDIIFWAHDRFGGYAQSGLLAEITPDKAFQDKLYPFTWDAVRYNGKLIAYPIAVEALSLIYNKDLLPNPPKTWEEIPALDKELKAKGKSALMFNLQEPYFTWPLIAADGGYAFKYENGKYDIKDVGVDNAGAKAGLTFLVDLIKNKHMNADTDYSIAEAAFNKGETAMTINGPWAWSNIDTSKVNYGVTVLPTFKGQPSKPFVGVLSAGINAASPNKELAKEFLENYLLTDEGLEAVNKDKPLGAVALKSYEEELVKDPRIAATMENAQKGEIMPNIPQMSAFWYAVRTAVINAASGRQTVDEALKDAQTNSSSENLYFQGGSEVQLVESGGGLVQPGGSLRLSCAASGFILDYYAIGWFRQAPGKEREGVLCIDASDDITYYADSVKGRFTISRDNAKNTVYLQMNSLKPEDTGVYYCATPIGLSSSCLLEYDYDYWGQGTLVTVSSGGSGGSGGSGGSASMKGGSWGGSKKTPPPVPPRTTSKGGSGGSGGSGGSKKTPPPVPPRTTSKGGSGGSGGSGGSDLNMPAYVKFNYMAEREDELSLIKGTKVIVMEKSSDGWWRGSYNGQVGWFPSNYVTEEGDSPLASGAGGSEGGGSEGGTSGATDLNMPAYVKFNYMAEREDELSLIKGTKVIVMEKSSDGWWRGSYNGQVGWFPSNYVTEEGDSPLGSMGMGEVQLLESGGGLVQPGGSLRLSCAASGTFDKINNMGWYRQAPGKQRDLVAQITPGGITDYADSVKGRFTISRDNSKNTLYLQMNSLRPEDTAVYYCNAEILKRAYIDVYVNYWGQGTLVTVSSEFPAGNHHHHHH

SEQ ID NO: 10 - protein, 735 aa, synthetic construct
MKIEEGKLVIWINGDKGYNGLAEVGKKFEKDTGIKVTVEHPDKLEEKFPQVAATGDGPDIIFWAHDRFGGYAQSGLLAEITPDKAFQDKLYPFTWDAVRYNGKLIAYPIAVEALSLIYNKDLLPNPPKTWEEIPALDKELKAKGKSALMFNLQEPYFTWPLIAADGGYAFKYENGKYDIKDVGVDNAGAKAGLTFLVDLIKNKHMNADTDYSIAEAAFNKGETAMTINGPWAWSNIDTSKVNYGVTVLPTFKGQPSKPFVGVLSAGINAASPNKELAKEFLENYLLTDEGLEAVNKDKPLGAVALKSYEEELVKDPRIAATMENAQKGEIMPNIPQMSAFWYAVRTAVINAASGRQTVDEALKDAQTNSSSENLYFQGGSGSASMKGGSWGGSKKTPPPVPPRTTSKGGSGGSGGSGGSKKTPPPVPPRTTSKGGSGGSGGSGGSDLNMPAYVKFNYMAEREDELSLIKGTKVIVMEKSSDGWWRGSYNGQVGWFPSNYVTEEGDSPLASGAGGSEGGGSEGGTSGATDLNMPAYVKFNYMAEREDELSLIKGTKVIVMEKSSDGWWRGSYNGQVGWFPSNYVTEEGDSPLGSMGEVQLMESGGGLVQAGGSLRLSCAASGRTFNNYAMGWFRRAPKGEREFVAAITRSGVRSGVSAIYGDSVKDRFTISRDNAKNTLYLQMNSLKPEDTAVYTCAASAIGSGALRRFEYDYSGQGTQVTVSSEFPAGNHHHHHH

SEQ ID NO: 11 - protein, 731 aa, synthetic construct
MKIEEGKLVIWINGDKGYNGLAEVGKKFEKDTGIKVTVEHPDKLEEKFPQVAATGDGPDIIFWAHDRFGGYAQSGLLAEITPDKAFQDKLYPFTWDAVRYNGKLIAYPIAVEALSLIYNKDLLPNPPKTWEEIPALDKELKAKGKSALMFNLQEPYFTWPLIAADGGYAFKYENGKYDIKDVGVDNAGAKAGLTFLVDLIKNKHMNADTDYSIAEAAFNKGETAMTINGPWAWSNIDTSKVNYGVTVLPTFKGQPSKPFVGVLSAGINAASPNKELAKEFLENYLLTDEGLEAVNKDKPLGAVALKSYEEELVKDPRIAATMENAQKGEIMPNIPQMSAFWYAVRTAVINAASGRQTVDEALKDAQTNSSSENLYFQGGSGSASMKGGSWGGSKKTPPPVPPRTTSKGGSGGSGGSGGSKKTPPPVPPRTTSKGGSGGSGGSGGSDLNMPAYVKFNYMAEREDELSLIKGTKVIVMEKSSDGWWRGSYNGQVGWFPSNYVTEEGDSPLASGAGGSEGGGSEGGTSGATDLNMPAYVKFNYMAEREDELSLIKGTKVIVMEKSSDGWWRGSYNGQVGWFPSNYVTEEGDSPLGSMGMGEVQLLESGGGLVQPGGSLRLSCAASGTFDKINNMGWYRQAPGKQRDLVAQITPGGITDYADSVKGRFTISRDNSKNTLYLQMNSLRPEDTAVYYCNAEILKRAYIDVYVNYWGQGTLVTVSSEFPAGNHHHHHH

SEQ ID NO: 12 - protein, 680 aa, synthetic construct
MKIEEGKLVIWINGDKGYNGLAEVGKKFEKDTGIKVTVEHPDKLEEKFPQVAATGDGPDIIFWAHDRFGGYAQSGLLAEITPDKAFQDKLYPFTWDAVRYNGKLIAYPIAVEALSLIYNKDLLPNPPKTWEEIPALDKELKAKGKSALMFNLQEPYFTWPLIAADGGYAFKYENGKYDIKDVGVDNAGAKAGLTFLVDLIKNKHMNADTDYSIAEAAFNKGETAMTINGPWAWSNIDTSKVNYGVTVLPTFKGQPSKPFVGVLSAGINAASPNKELAKEFLENYLLTDEGLEAVNKDKPLGAVALKSYEEELVKDPRIAATMENAQKGEIMPNIPQMSAFWYAVRTAVINAASGRQTVDEALKDAQTNSSSENLYFQGGSASMSEEKPKEGVKTENDHINLKVAGQDGSVVQFKIKRHTPLSKLMKAYCERQGLSMRQIRFRFDGQPINETDTPAQLEMEDEDTIDVFQQQTVVGGSGGSGGSGGSMSEEKPKEGVKTENDHINLKVAGQDGSVVQFKIKRHTPLSKLMKAYCERQGLSMRQIRFRFDGQPINETDTPAQLEMEDEDTIDVFQQQTVVGGSGGSGGSGGSKVDVIDLTIESSSDEEEDPPAKRGGSGGSGGRGGSKVDVIDLTIESSSDEEEDPPAKRGAMRCWGGSGGSGGSGGSMGEFPAGNHHHHHH

SEQ ID NO: 13 - protein, 944 aa, synthetic construct
MKIEEGKLVIWINGDKGYNGLAEVGKKFEKDTGIKVTVEHPDKLEEKFPQVAATGDGPDIIFWAHDRFGGYAQSGLLAEITPDKAFQDKLYPFTWDAVRYNGKLIAYPIAVEALSLIYNKDLLPNPPKTWEEIPALDKELKAKGKSALMFNLQEPYFTWPLIAADGGYAFKYENGKYDIKDVGVDNAGAKAGLTFLVDLIKNKHMNADTDYSIAEAAFNKGETAMTINGPWAWSNIDTSKVNYGVTVLPTFKGQPSKPFVGVLSAGINAASPNKELAKEFLENYLLTDEGLEAVNKDKPLGAVALKSYEEELVKDPRIAATMENAQKGEIMPNIPQMSAFWYAVRTAVINAASGRQTVDEALKDAQTNSSSENLYFQGGSEVQLMESGGGLVQAGGSLRLSCAASGRTFNNYAMGWFRRAPKGEREFVAAITRSGVRSGVSAIYGDSVKDRFTISRDNAKNTLYLQMNSLKPEDTAVYTCAASAIGSGALRRFEYDYSGQGTQVTVSSGGSGGSGGSGGSASMSEEKPKEGVKTENDHINLKVAGQDGSVVQFKIKRHTPLSKLMKAYCERQGLSMRQIRFRFDGQPINETDTPAQLEMEDEDTIDVFQQQTVVGGSGGSGGSGGSMSEEKPKEGVKTENDHINLKVAGQDGSVVQFKIKRHTPLSKLMKAYCERQGLSMRQIRFRFDGQPINETDTPAQLEMEDEDTIDVFQQQTVVGGSGGSGGSGGSKVDVIDLTIESSSDEEEDPPAKRGGSGGSGGRGGSKVDVIDLTIESSSDEEEDPPAKRGAMRCWGGSGGSGGSGGSMGMGEVQLLESGGGLVQPGGSLRLSCAASGTFDKINNMGWYRQAPGKQRDLVAQITPGGITDYADSVKGRFTISRDNSKNTLYLQMNSLRPEDTAVYYCNAEILKRAYIDVYVNYWGQGTLVTVSSEFPAGNHHHHHH

SEQ ID NO: 14 - protein, 601 aa, synthetic construct
MEGISIYTSDNYTEEMGSGDYDSMKEPCFREENANFNKIFLPTIYSIIFLTGIVGNGLVILVMGYQKKLRSMTDKYRLHLSVADLLFVITLPFWAVDAVANWYFGNFLCKAVHVIYTVNLYSSVLILAFISLDRYLAIVHATNSQRPRKLLAEKVVYVGVWIPALLLTIPDFIFANVSEADDRYICDRFYPNDLWVVVFQFQHIMVGLILPGIVILSCYCIIISKLSHSKGHQKRKALKTTVILILAFFACWLPYYIGISIDSFILLEIIKQGCEFENTVHKWISITEALAFFHCCLNPILYAFLGAKFKTSAQHALTSVSRGSSLKILSKGKRGGHSSVSTESESSSFHSSGGSGGSGGSGGSMKVSKGEEDNMAIIKEFMRFKVHMEGSVNGHEFEIEGEGEGRPYEGTQTAKLKVTKGGPLPFAWDILSPQFMYGSKAYVKHPADIPDYLKLSFPEGFKWERVMNFEDGGVVTVTQDSSLQDGEFIYKVKLRGTNFPSDGPVMQKKTMGWEASSERMYPEDGALKGEIKQRLKLKDGGHYDAEVKTTYKAKKPVQLPGAYNVNIKLDITSHNEDYTIVEQYERAEGRHSTGGMDELYK

SEQ ID NO: 15 - protein, 691 aa, synthetic construct
MEQRGQNAPAASGARKRHGPGPREARGARPGLRVPKTLVLVVAAVLLLVSAESALITQQDLAPQQRAAPQQKRSSPSEGLCPPGHHISEDGRDCISCKYGQDYSTHWNDLLFCLRCTRCDSGEVELSPCTTTRNTVCQCEEGTFREEDSPEMCRKCRTGCPRGMVKVGDCTPWSDIECVHKESGTKHSGEAPAVEETVTSSPGTPASPCSLSGIIIGVTVAAVVLIVAVFVCKSLLWKKVLPYLKGICSGGGGDPERVDRSSQRPGAEDNVLNEIVSILQPTQVPEQEMEVQEPAEPTGVNMLSPGESEHLLEPAEAERSQRRRLLVPANEGDPTETLRQCFDDFADLVPFDSWEPLMRKLGLMDNEIKVAKAEAAGHRDTLYTMLIKWVNKTGRDASVHTLLDALETLGERLAKQKIEDHLLSSGKFMYLEGNADSAMSGGSGGSGGSGGSMVSKGEELFTGVVPILVELDGDVNGHKFSVSGEGEGDATYGKLTLKFICTTGKLPVPWPTLVTTLTYGVQCFSRYPDHMKQHDFFKSAMPEGYVQERTIFFKDDGNYKTRAEVKFEGDTLVNRIELKGIDFKEDGNILGHKLEYNYNSHNVYIMADKQKNGIKVNFKIRHNIEDGSVQLADHYQQNTPIGDGPVLLPDNHYLSTQSALSKDPNEKRDHMVLLEFVTAAGITLGMDELYK

SEQ ID NO: 16 - protein, 184 aa, synthetic construct
MKGGSWGGSKKTPPPVPPRTTSKGGSGGSGGSGGSKKTPPPVPPRTTSKASGAGGSEVQLMESGGGLVQAGGSLRLSCAASGRTFNNYAMGWFRRAPKGEREFVAAITRSGVRSGVSAIYGDSVKDRFTISRDNAKNTLYLQMNSLKPEDTAVYTCAASAIGSGALRRFEYDYSGQGTQVTVSS

SEQ ID NO: 17 - protein, 274 aa, synthetic construct
DLNMPAYVKFNYMAEREDELSLIKGTKVIVMEKSSDGWWRGSYNGQVGWFPSNYVTEEGDSPLASGAGGSEGGGSEGGTSGATDLNMPAYVKFNYMAEREDELSLIKGTKVIVMEKSSDGWWRGSYNGQVGWFPSNYVTEEGDSPLGSMGMGEVQLLESGGGLVQPGGSLRLSCAASGTFDKINNMGWYRQAPGKQRDLVAQITPGGITDYADSVKGRFTISRDNSKNTLYLQMNSLRPEDTAVYYCNAEILKRAYIDVYVNYWGQGTLVTVSS

SEQ ID NO: 18 - protein, 208 aa, synthetic construct
MKGGSWGGSKKTPPPVPPRTTSKGGSGGSGGSGGSKKTPPPVPPRTTSKGGSGGSGGSGGSDLNMPAYVKFNYMAEREDELSLIKGTKVIVMEKSSDGWWRGSYNGQVGWFPSNYVTEEGDSPLASGAGGSEGGGSEGGTSGATDLNMPAYVKFNYMAEREDELSLIKGTKVIVMEKSSDGWWRGSYNGQVGWFPSNYVTEEGDSPLG

SEQ ID NO: 19 - protein, 196 aa, synthetic construct
MSEEKPKEGVKTENDHINLKVAGQDGSVVQFKIKRHTPLSKLMKAYCERQGLSMRQIRFRFDGQPINETDTPAQLEMEDEDTIDVFQQQTVVGGSGGSGGSGGSMSEEKPKEGVKTENDHINLKVAGQDGSVVQFKIKRHTPLSKLMKAYCERQGLSMRQIRFRFDGQPINETDTPAQLEMEDEDTIDVFQQQTVV

SEQ ID NO: 20 - protein, 128 aa, synthetic construct
EVQLMESGGGLVQAGGSLRLSCAASGRTFNNYAMGWFRRAPKGEREFVAAITRSGVRSGVSAIYGDSVKDRFTISRDNAKNTLYLQMNSLKPEDTAVYTCAASAIGSGALRRFEYDYSGQGTQVTVSS

SEQ ID NO: 21 - protein, 124 aa, synthetic construct
MGEVQLLESGGGLVQPGGSLRLSCAASGTFDKINNMGWYRQAPGKQRDLVAQITPGGITDYADSVKGRFTISRDNSKNTLYLQMNSLRPEDTAVYYCNAEILKRAYIDVYVNYWGQGTLVTVSS

SEQ ID NO: 22 - protein, 127 aa, synthetic construct
EVQLVESGGGLVQAGGSLRLSCAASGRTFSSYAMGWFRQAPGKEREFVVAINWSSGSTYYADSVKGRFTISRDNAKNTMYLQMNSLKPEDTAVYYCAAGYQINSGNYNFKDYEYDYWGQGTQVTVSS

SEQ ID NO: 23 - protein, 125 aa, synthetic construct
EVQLVESGGGLVQPGGSLRLSCAASGFILDYYAIGWFRQAPGKEREGVLCIDASDDITYYADSVKGRFTISRDNAKNTVYLQMNSLKPEDTGVYYCATPIGLSSSCLLEYDYDYWGQGTLVTVSS

SEQ ID NO: 24 - protein, 477 aa, synthetic construct
EVQLMESGGGLVQAGGSLRLSCAASGRTFNNYAMGWFRRAPKGEREFVAAITRSGVRSGVSAIYGDSVKDRFTISRDNAKNTLYLQMNSLKPEDTAVYTCAASAIGSGALRRFEYDYSGQGTQVTVSSGGSGGSGGSGGSASMKGGSWGGSKKTPPPVPPRTTSKGGSGGSGGSGGSKKTPPPVPPRTTSKGGSGGSGGSGGSDLNMPAYVKFNYMAEREDELSLIKGTKVIVMEKSSDGWWRGSYNGQVGWFPSNYVTEEGDSPLASGAGGSEGGGSEGGTSGATDLNMPAYVKFNYMAEREDELSLIKGTKVIVMEKSSDGWWRGSYNGQVGWFPSNYVTEEGDSPLGSMGMGEVQLLESGGGLVQPGGSLRLSCAASGTFDKINNMGWYRQAPGKQRDLVAQITPGGITDYADSVKGRFTISRDNSKNTLYLQMNSLRPEDTAVYYCNAEILKRAYIDVYVNYWGQGTLVTVSS

SEQ ID NO: 25 - protein, 552 aa, synthetic construct
EVQLMESGGGLVQAGGSLRLSCAASGRTFNNYAMGWFRRAPKGEREFVAAITRSGVRSGVSAIYGDSVKDRFTISRDNAKNTLYLQMNSLKPEDTAVYTCAASAIGSGALRRFEYDYSGQGTQVTVSSGGSGGSGGSGGSASMSEEKPKEGVKTENDHINLKVAGQDGSVVQFKIKRHTPLSKLMKAYCERQGLSMRQIRFRFDGQPINETDTPAQLEMEDEDTIDVFQQQTVVGGSGGSGGSGGSMSEEKPKEGVKTENDHINLKVAGQDGSVVQFKIKRHTPLSKLMKAYCERQGLSMRQIRFRFDGQPINETDTPAQLEMEDEDTIDVFQQQTVVGGSGGSGGSGGSKVDVIDLTIESSSDEEEDPPAKRGGSGGSGGRGGSKVDVIDLTIESSSDEEEDPPAKRGAMRCWGGSGGSGGSGGSMGMGEVQLLESGGGLVQPGGSLRLSCAASGTFDKINNMGWYRQAPGKQRDLVAQITPGGITDYADSVKGRFTISRDNSKNTLYLQMNSLRPEDTAVYYCNAEILKRAYIDVYVNYWGQGTLVTVSS

SEQ ID NO: 26 - protein, 453 aa, synthetic construct
  source 1..453: note = FADD with a BFP tag fused to the C-terminal
MSELIKENMHMKLYMEGTVDNHHFKCTSEGEGKPYEGTQTMRIKVVEGGPLPFAFDILATSFLYGSKTFINHTQGIPDFFKQSFPEGFTWERVTTYEDGGVLTATQDTSLQDGCLIYNVKIRGVNFTSNGPVMQKKTLGWEAFTETLYPADGGLEGRNDMALKLVGGSHLIANIKTTYRSKKPAKNLKMPGVYYVDYRLERIKEANNETYVEQHEVAVARYCDLPSKLGHKLNGGSGGSGGSGGSMDPFLVLLHSVSSSLSSSELTELKFLCLGRVGKRKLERVQSGLDLFSMLLEQNDLEPGHTELLRELLASLRRHDLLRRVDDFEAGAAAGAAPGEEDLCAAFNVICDNVGKDWRRLARQLKVSDTKIDSIEDRYPRNLTERVRESLRIWKNTEKENATVAHLVGALRSCQMNLVADLVQEVQQARDLQNRSGAMSPMSWNSDASTSEAS

SEQ ID NO: 27 - protein, 778 aa, synthetic construct
  source 1..778: note = Fusion of CN, P1S1 and DN
MKIEEGKLVIWINGDKGYNGLAEVGKKFEKDTGIKVTVEHPDKLEEKFPQVAATGDGPDIIFWAHDRFGGYAQSGLLAEITPDKAFQDKLYPFTWDAVRYNGKLIAYPIAVEALSLIYNKDLLPNPPKTWEEIPALDKELKAKGKSALMFNLQEPYFTWPLIAADGGYAFKYENGKYDIKDVGVDNAGAKAGLTFLVDLIKNKHMNADTDYSIAEAAFNKGETAMTINGPWAWSNIDTSKVNYGVTVLPTFKGQPSKPFVGVLSAGINAASPNKELAKEFLENYLLTDEGLEAVNKDKPLGAVALKSYEEELVKDPRIAATMENAQKGEIMPNIPQMSAFWYAVRTAVINAASGRQTVDEALKDAQTNSSSENLYFQGGSEVQLMESGGGLVQAGGSLRLSCAASGRTFNNYAMGWFRRAPKGEREFVAAITRSGVRSGVSAIYGDSVKDRFTISRDNAKNTLYLQMNSLKPEDTAVYTCAASAIGSGALRRFEYDYSGQGTQVTVSSGGSGGSGGSGGSASMKGGSWGGSKKTPPPVPPRTTSKASGAGGSEGGGSEGGTSGATDLNMPAYVKFNYMAEREDELSLIKGTKVIVMEKSSDGWWRGSYNGQVGWFPSNYVTEEGDSPLGGSGGSGGSGGSMGMGEVQLLESGGGLVQPGGSLRLSCAASGTFDKINNMGWYRQAPGKQRDLVAQITPGGITDYADSVKGRFTISRDNSKNTLYLQMNSLRPEDTAVYYCNAEILKRAYIDVYVNYWGQGTLVTVSSEFPAGNHHHHHH

SEQ ID NO: 28 - protein, 869 aa, synthetic construct
  source 1..869: note = Fusion of CN, P2S2 (mutant) and DN with MBP tag and His6 tag fused to the N-terminal and C-terminal respectively
MKIEEGKLVIWINGDKGYNGLAEVGKKFEKDTGIKVTVEHPDKLEEKFPQVAATGDGPDIIFWAHDRFGGYAQSGLLAEITPDKAFQDKLYPFTWDAVRYNGKLIAYPIAVEALSLIYNKDLLPNPPKTWEEIPALDKELKAKGKSALMFNLQEPYFTWPLIAADGGYAFKYENGKYDIKDVGVDNAGAKAGLTFLVDLIKNKHMNADTDYSIAEAAFNKGETAMTINGPWAWSNIDTSKVNYGVTVLPTFKGQPSKPFVGVLSAGINAASPNKELAKEFLENYLLTDEGLEAVNKDKPLGAVALKSYEEELVKDPRIAATMENAQKGEIMPNIPQMSAFWYAVRTAVINAASGRQTVDEALKDAQTNSSSENLYFQGGSEVQLMESGGGLVQAGGSLRLSCAASGRTFNNYAMGWFRRAPKGEREFVAAITRSGVRSGVSAIYGDSVKDRFTISRDNAKNTLYLQMNSLKPEDTAVYTCAASAIGSGALRRFEYDYSGQGTQVTVSSGGSGGSGGSGGSASMKGGSWGGSKKTAAAVAARTTSKGGSGGSGGSGGSKKTAAAVAARTTSKGGSGGSGGSGGSDLNMPAYVKFNYMAEREDELSLIKGTKVIVMEKSSDGWWRGSYNGQVGWFPSNYVTEEGDSPLASGAGGSEGGGSEGGTSGATDLNMPAYVKFNYMAEREDELSLIKGTKVIVMEKSSDGWWRGSYNGQVGWFPSNYVTEEGDSPLGSMGMGEVQLLESGGGLVQPGGSLRLSCAASGTFDKINNMGWYRQAPGKQRDLVAQITPGGITDYADSVKGRFTISRDNSKNTLYLQMNSLRPEDTAVYYCNAEILKRAYIDVYVNYWGQGTLVTVSSEFPAGNHHHHHH